European Patent Application EP 4 703 381 A1, published March 4, 2026. Title: ANTIBODIES AGAINST ICAM-1 AND APPLICATIONS THEREOF. Applicant: Institució Catalana de Recerca i Estudis Avançats. The sequence listing filed with the application follows.

SEQUENCE LISTING (32 sequences)

SEQ ID NO: 1 - protein, 128 aa, synthetic construct
QVQLVESGGGLVQPGGSLRLSCSASGFTFSSYAMHWVRQAPGKGLEYVSAISSNGGSTYYADSVKGRFTISRDNSKNTLYLQMSSLRAEDTAVYYCVKGSNTKQWLAGGYYYYGMDVWGQGTTVTVSS

SEQ ID NO: 2 - protein, 107 aa, synthetic construct
AIRMTQSPSSVSASVGDRVTITCRASQGISSWLAWYQQKPGKAPKLLIYAASSLQSGVPSRFSGSGSGTDFTLTISSLQPEDFATYYCQQANSFPYTFGQGTKVDIK

SEQ ID NO: 3 - protein, 123 aa, synthetic construct
QMQLVQSGGGVVQPGRSLRLSCAASGLTFSSYGMHWVRQAPGKGLEWVAVISYDGSNKYYADSVKGRFTISRDNSKNTLYLQMNSLRAEDTAVYYCAKDFYNWNDWHDAFDIWGQGTMVTVSS

SEQ ID NO: 4 - protein, 107 aa, synthetic construct
DIVMTQSPSSLSASVGDSVTITCRASQDISNYLAWYQQKPGKAPKLLIFAASTLQSGVPSRFSGSGSGTDFALTISSLQPEDVASYYCQKYNHVPQTFGPGTQVDIK

SEQ ID NO: 5 - protein, 8 aa, synthetic construct
GFTFSSYA

SEQ ID NO: 6 - protein, 8 aa, synthetic construct
ISSNGGST

SEQ ID NO: 7 - protein, 21 aa, synthetic construct
VKGSNTKQWLAGGYYYYGMDV

SEQ ID NO: 8 - protein, 6 aa, synthetic construct
QGISSW

SEQ ID NO: 9 - skipped

SEQ ID NO: 10 - protein, 9 aa, synthetic construct
QQANSFPYT

SEQ ID NO: 11 - protein, 8 aa, synthetic construct
GLTFSSYG

SEQ ID NO: 12 - protein, 8 aa, synthetic construct
ISYDGSNK

SEQ ID NO: 13 - protein, 16 aa, synthetic construct
AKDFYNWNDWHDAFDI

SEQ ID NO: 14 - protein, 6 aa, synthetic construct
QDISNY

SEQ ID NO: 15 - skipped

SEQ ID NO: 16 - protein, 9 aa, synthetic construct
QKYNHVPQT

SEQ ID NO: 17 - protein, 25 aa, synthetic construct
QVQLVESGGGLVQPGGSLRLSCSAS

SEQ ID NO: 18 - protein, 17 aa, synthetic construct
MHWVRQAPGKGLEYVSA

SEQ ID NO: 19 - protein, 38 aa, synthetic construct
YYADSVKGRFTISRDNSKNTLYLQMSSLRAEDTAVYYC

SEQ ID NO: 20 - protein, 11 aa, synthetic construct
WGQGTTVTVSS

SEQ ID NO: 21 - protein, 26 aa, synthetic construct
AIRMTQSPSSVSASVGDRVTITCRAS

SEQ ID NO: 22 - protein, 17 aa, synthetic construct
LAWYQQKPGKAPKLLIY

SEQ ID NO: 23 - protein, 36 aa, synthetic construct
SLQSGVPSRFSGSGSGTDFTLTISSLQPEDFATYYC

SEQ ID NO: 24 - protein, 10 aa, synthetic construct
FGQGTKVDIK

SEQ ID NO: 25 - protein, 25 aa, synthetic construct
QMQLVQSGGGVVQPGRSLRLSCAAS

SEQ ID NO: 26 - protein, 17 aa, synthetic construct
MHWVRQAPGKGLEWVAV

SEQ ID NO: 27 - protein, 38 aa, synthetic construct
YYADSVKGRFTISRDNSKNTLYLQMNSLRAEDTAVYYC

SEQ ID NO: 28 - protein, 11 aa, synthetic construct
WGQGTMVTVSS

SEQ ID NO: 29 - protein, 26 aa, synthetic construct
DIVMTQSPSSLSASVGDSVTITCRAS

SEQ ID NO: 30 - protein, 17 aa, synthetic construct
LAWYQQKPGKAPKLLIF

SEQ ID NO: 31 - protein, 36 aa, synthetic construct
TLQSGVPSRFSGSGSGTDFALTISSLQPEDVASYYC

SEQ ID NO: 32 - protein, 10 aa, synthetic construct
FGPGTQVDIK